European Patent Specification EP 3 453 395 B1, published October 18, 2023. Title: TENERICUTES FOR USE IN THE TREATMENT OR PREVENTION OF AN INFLAMMATORY DISORDER OF THE DIGESTIVE SYSTEM. Applicant: Deutsches Rheuma-Forschungszentrum Berlin. The sequence listing filed with the application follows.

SEQUENCE LISTING (4 sequences)

SEQ ID NO: 1 - DNA, 21 bp, Mus musculus
cacagctcacggcaccggaga

SEQ ID NO: 2 - DNA, 23 bp, Mus musculus
gctgtactgtgtgtccaggctcc

SEQ ID NO: 3 - DNA, 23 bp, Mus musculus
cgaggtcacaggagaagggacgc

SEQ ID NO: 4 - DNA, 22 bp, Mus musculus
ccgaaagagtctctgcagctcc